European Patent Application EP 4 775 664 A1, published July 15, 2026. Title: STRAIN OF DUGANELLA SP., EXOPOLYSACCHARIDE PRODUCED THEREBY, AND USE. Applicant: Nanjing Southern Element Biotechnology Co., Ltd. The sequence listing filed with the application follows.

SEQUENCE LISTING (1 sequence)

SEQ ID NO: 1 - DNA, 1532 bp, Duganella sp.
  source 1..1532: mol_type = genomic DNA; note = 16S sequence
taaactgaagagtttgatcctggctcagattgaacgctggcggcatgccttacacatgcaagtcgaacggcagcgcggggcaacctggcggcgagtggcgaacgggtgagtaatatatcggaacgtaccctggagtgggggataacgtagcgaaagttacgctaataccgcatacgatctcaggatgaaagcaggggaccgcaaggccttgtgctcctggagcggccgatatctgattagctagttggtagggtaaaagcctaccaaggcatcgatcagtagctggtctgagaggacgaccagccacactggaactgagacacggtccagactcctacgggaggcagcagtggggaattttggacaatgggcgcaagcctgatccagcaatgccgcgtgagtgaagaaggccttcgggttgtaaagctcttttgtcagggaagaaacggtgagggctaatatcccttgctaatgacggtacctgaagaataagcaccggctaactacgtgccagcagccgcggtaatacgtagggtgcaagcgttaatcggaattactgggcgtaaagcgtgcgcaggcggttttgtaagtttgtcgtgaaatccccgggctcaacctgggaatggcgatgaagactgcaaggctagagtttggcagaggggggtagaattccacgtgtagcagtgaaatgcgtagatatgtggaggaacaccgatggcgaaggcagccccctgggtcaaaactgacgctcatgcacgaaagcgtggggagcaaacaggattagataccctggtagtccacgccctaaacgatgtctactagttgtcgggtcttaattgacttggtaacgcagctaacgcgtgaagtagaccgcctggggagtacggtcgcaagattaaaactcaaaggaattgacggggacccgcacaagcggtggatgatgtggattaattcgatgcaacgcgaaaaaccttacctacccttgacatggatggaatcccggagagatttgggagtgcccgaaagggaaccatcacacaggtgctgcatggctgtcgtcagctcgtgtcgtgagatgttgggttaagtcccgcaacgagcgcaacccttgtcattagttgctacgaaagagcactctaatgagactgccggtgacaaaccggaggaaggtggggatgacgtcaagtcctcatggcccttatgggtagggcttcacacgtcatacaatggtacatacagagggccgccaacccgcgagggggagctaatcccagaaagtgtatcgtagtccggattgtagtctgcaactcgactgcatgaagttggaatcgctagtaatcgcggatcagcatgtcgcggtgaatacgttcccgggtcttgtacacaccgcccgtcacaccatgggagcgggttttaccagaagtaggtagcttaaccgcaaggagggcgcttaccacggtaggattcgtgactggggtgaagtcgtaacaaggtagccgtatcggaaggtgcggctggatcacctcctttct